European Patent Specification EP 3 643 302 B1, published September 20, 2023. Title: Composition comprising sesquiterpene derivatives or as active ingredients for preventing and treating muscle diseases. Applicant: Industry-Academic Cooperation Foundation, Yonsei University. The sequence listing filed with the application follows.

SEQUENCE LISTING (6 sequences)

SEQ ID NO: 1 - DNA, 20 bp, Artificial Sequence
  MaFbx_F primer
gtccagagagtcggcaagtc

SEQ ID NO: 2 - DNA, 20 bp, Artificial Sequence
  MaFbx_R primer
gtcggtgatcgtgagacctt

SEQ ID NO: 3 - DNA, 20 bp, Artificial Sequence
  MuRF1_F primer
acatctactgtctcacgtgt

SEQ ID NO: 4 - DNA, 20 bp, Artificial Sequence
  MuRF1_R primer
tgtccttggaagatgctttg

SEQ ID NO: 5 - DNA, 20 bp, Artificial Sequence
  GAPDH_F primer
gtgatggcatggactgtggt

SEQ ID NO: 6 - DNA, 20 bp, Artificial Sequence
  GAPDH_R primer
ggagccaaaagggtcatcat